European Patent Specification EP 3 105 341 B1, published September 3, 2025. Title: Screening Assay for Gibberellin Inhibitors or Analogs. Applicant: MAX-PLANCK-GESELLSCHAFT zur FÖRDERUNG der WISSENSCHAFTEN e.V. Eberhard Karls Universität Tübingen. The sequence listing filed with the application follows.

SEQUENCE LISTING (26 sequences)

SEQ ID NO: 1 - protein, 939 aa, Photinus pyralis
MSGYVNNPEATNALIDKDGWLHSGDIAYWDEDEHFFIVDRLKSLIKYKGYQVAPAELESILLQHPNIFDAGVAGLPDDDAGELPAAVVVLEHGKTMTEKEIVDYVASQVTTAKKLRGGVVFVDEVPKGLTGKLDARKIREILIKAKKGGKIAVGGGGGGGAGGNEVNLNECKRIVPLNTWVLISNFKLAYKVLRRPDGSFNRDLAEFLDRKVPANSFPLDGVFSFDHVDSTTNLLTRIYQPASLLHQTRHGTLELTKPLSTTEIVPVLIFFHGGSFTHSSANSAIYDTFCRRLVTICGVVVVSVDYRRSPEHRYPCAYDDGWNALNWVKSRVWLQSGKDSNVYVYLAGDSSGGNIAHNVAVRATNEGVKVLGNILLHPMFGGQERTQSEKTLDGKYFVTIQDRDWYWRAYLPEGEDRDHPACNPFGPRGQSLKGVNFPKSLVVVAGLDLVQDWQLAYVDGLKKTGLEVNLLYLKQATIGFYFLPNNDHFHCLMEELNKFVHSIEDSQSKSSPVLLTPGGGGGGGEDAKNIKKGPAPFYPLEDGTAGEQLHKAMKRYALVPGTIAFTDAHIEVDITYAEYFEMSVRLAEAMKRYGLNTNHRIVVCSENSLQFFMPVLGALFIGVAVAPANDIYNERELLNSMGISQPTVVFVSKKGLQKILNVQKKLPIIQKIIIMDSKTDYQGFQSMYTFVTSHLPPGFNEYDFVPESFDRDKTIALIMNSSGSTGLPKGVALPHRTACVRFSHARDPIFGNQIIPDTAILSVVPFHHGFGMFTTLGYLICGFRVVLMYRFEEELFLRSLQDYKIQSALLVPTLFSFFAKSTLIDKYDLSNLHEIASGGAPLSKEVGEAVAKRFHLPGIRQGYGLTETTSAILITPEGDDKPGAVGKVVPFFEAKVVDLDTGKTLGVNQRGELCVRGPMIMSGYVNNPEATNALIDKDG

SEQ ID NO: 2 - protein, 1179 aa, Artificial Sequence
  GID1B sensor peptide
MSGYVNNPEATNALIDKDGWLHSGDIAYWDEDEHFFIVDRLKSLIKYKGYQVAPAELESILLQHPNIFDAGVAGLPDDDAGELPAAVVVLEHGKTMTEKEIVDYVASQVTTAKKLRGGVVFVDEVPKGLTGKLDARKIREILIKAKKGGKIAVGGGGGGGAGGNEVNLNECKRIVPLNTWVLISNFKLAYKVLRRPDGSFNRDLAEFLDRKVPANSFPLDGVFSFDHVDSTTNLLTRIYQMSGYVNNPEATNALIDKDGWLHSGDIAYWDEDEHFFIVDRLKSLIKYKGYQVAPAELESILLQHPNIFDAGVAGLPDDDAGELPAAVVVLEHGKTMTEKEIVDYVASQVTTAKKLRGGVVFVDEVPKGLTGKLDARKIREILIKAKKGGKIAVGGGGGGGAGGNEVNLNECKRIVPLNTWVLISNFKLAYKVLRRPDGSFNRDLAEFLDRKVPANSFPLDGVFSFDHVDSTTNLLTRIYQPASLLHQTRHGTLELTKPLSTTEIVPVLIFFHGGSFTHSSANSAIYDTFCRRLVTICGVVVVSVDYRRSPEHRYPCAYDDGWNALNWVKSRVWLQSGKDSNVYVYLAGDSSGGNIAHNVAVRATNEGVKVLGNILLHPMFGGQERTQSEKTLDGKYFVTIQDRDWYWRAYLPEGEDRDHPACNPFGPRGQSLKGVNFPKSLVVVAGLDLVQDWQLAYVDGLKKTGLEVNLLYLKQATIGFYFLPNNDHFHCLMEELNKFVHSIEDSQSKSSPVLLTPGGGGGGGEDAKNIKKGPAPFYPLEDGTAGEQLHKAMKRYALVPGTIAFTDAHIEVDITYAEYFEMSVRLAEAMKRYGLNTNHRIVVCSENSLQFFMPVLGALFIGVAVAPANDIYNERELLNSMGISQPTVVFVSKKGLQKILNVQKKLPIIQKIIIMDSKTDYQGFQSMYTFVTSHLPPGFNEYDFVPESFDRDKTIALIMNSSGSTGLPKGVALPHRTACVRFSHARDPIFGNQIIPDTAILSVVPFHHGFGMFTTLGYLICGFRVVLMYRFEEELFLRSLQDYKIQSALLVPTLFSFFAKSTLIDKYDLSNLHEIASGGAPLSKEVGEAVAKRFHLPGIRQGYGLTETTSAILITPEGDDKPGAVGKVVPFFEAKVVDLDTGKTLGVNQRGELCVRGPMIMSGYVNNPEATNALIDKDG

SEQ ID NO: 3 - DNA, 2820 bp, Artificial Sequence
  GID1B sensor nucleotide sequence
atgtccggttatgtaaacaatccggaagcgaccaacgccttgattgacaaggatggatggctacattctggagacatagcttactgggacgaagacgaacacttcttcatcgttgaccgcctgaagtctctgattaagtacaaaggctatcaggtggctcccgctgaattggaatccatcttgctccaacaccccaacatcttcgacgcaggtgtcgcaggtcttcccgacgatgacgccggtgaacttcccgccgccgttgttgttttggagcacggaaagacgatgacggaaaaagagatcgtggattacgtcgccagtcaagtaacaaccgcgaaaaagttgcgcggaggagttgtgtttgtggacgaagtaccgaaaggtcttaccggaaaactcgacgcaagaaaaatcagagagatcctcataaaggccaagaagggcggaaagatcgccgtgggtggcgggggtggcggaggagctggtggtaacgaagtcaaccttaacgaatgcaagagaattgtcccactcaacacatgggtcctcatttccaatttcaagcttgcttacaaagtcctccgtcgccctgacggttctttcaaccgcgacctcgccgagttccttgaccgtaaagttcccgccaactctttccccctcgacggcgttttctccttcgaccacgtcgactcaacaactaaccttctcaccagaatctaccaacctgcgtctctccttcatcagacccgtcacggaaccctcgagctaaccaaacctctcagtactacagagatcgtccctgttctcattttcttccatggaggcagcttcactcattcctccgccaatagtgctatctacgacactttctgccgacgccttgtcaccatttgcggtgttgttgttgtctctgttgattaccggagatcccctgagcatcgctacccttgtgcttacgacgatggatggaacgctctcaactgggtcaagtccagagtctggcttcagagtggtaaagactccaatgtttatgtttatttggctggagatagctctggaggcaacattgctcacaatgtcgctgtcagagctaccaatgaaggagtcaaagtgttggggaacattcttcttcatccaatgtttggtggacaggagaggactcagtctgagaagacccttgatggcaaatactttgtgactatacaagatcgagattggtattggagggcttatctaccggaaggtgaagatagagatcatccagcatgtaatccctttggcccgagaggtcaaagccttaaaggagtcaactttccaaagagtcttgttgttgtcgctggtttagatcttgttcaagattggcaattagcctatgtggatgggcttaagaagactggtcttgaagtcaatcttttgtatttgaaacaagctaccattggcttttacttcttgcctaacaatgatcactttcattgtcttatggaagagttgaataagtttgtgcactccatagaggattctcaaagcaagtcaagtcctgtgcttcttactcctggtggaggcggaggcggaggcgaagacgccaaaaacataaagaaaggcccggcgccattctatccgctggaagatggaaccgctggagagcaactgcataaggctatgaagagatacgccctggttcctggaacaattgcttttacagatgcacatatcgaggtggacatcacttacgctgagtacttcgaaatgtccgttcggttggcagaagctatgaaacgatatgggctgaatacaaatcacagaatcgtcgtatgcagtgaaaactctcttcaattctttatgccggtgttgggcgcgttatttatcggagttgcagttgcgcccgcgaacgacatttataatgaacgtgaattgctcaacagtatgggcatttcgcagcctaccgtggtgttcgtttccaaaaaggggttgcaaaaaattttgaacgtgcaaaaaaagctcccaatcatccaaaaaattattatcatggattctaaaacggattaccagggatttcagtcgatgtacacgttcgtcacatctcatctacctcccggttttaatgaatacgattttgtgccagagtccttcgatagggacaagacaattgcactgatcatgaactcctctggatctactggtctgcctaaaggtgtcgctctgcctcatagaactgcctgcgtgagattctcgcatgccagagatcctatttttggcaatcaaatcattccggatactgcgattttaagtgttgttccattccatcacggttttggaatgtttactacactcggatatttgatatgtggatttcgagtcgtcttaatgtatagatttgaagaagagctgtttctgaggagccttcaggattacaagattcaaagtgcgctgctggtgccaaccctattctccttcttcgccaaaagcactctgattgacaaatacgatttatctaatttacacgaaattgcttctggtggcgctcccctctctaaggaagtcggggaagcggttgccaagaggttccatctgccaggtatcaggcaaggatatgggctcactgagactacatcagctattctgattacacccgagggggatgataaaccgggcgcggtcggtaaagttgttccattttttgaagcgaaggttgtggatctggataccgggaaaacgctgggcgttaatcaaagaggcgaactgtgtgtgagaggtcctatgattatgtccggttatgtaaacaatccggaagcgaccaacgccttgattgacaaggatggataa

SEQ ID NO: 4 - DNA, 21 bp, Artificial Sequence
  Primer for GID1b cDNA amplification
atggctggtggtaacgaagtc

SEQ ID NO: 5 - DNA, 20 bp, Artificial Sequence
  Primer for GID1b cDNA amplification
ctaaggagtaagaagcacag

SEQ ID NO: 6 - DNA, 23 bp, Artificial Sequence
  Primer for amplification of C-terminal domain of firefly luciferase
atgtccggttatgtaaacaatcc

SEQ ID NO: 7 - DNA, 53 bp, Artificial Sequence
  Primer for amplification of C-terminal domain of firefly luciferase with linker
gacttcgttaccaccagctcctccgccacccccgccacccacggcgatctttc

SEQ ID NO: 8 - DNA, 26 bp, Artificial Sequence
  Primer for addition of linker to GID1b cDNA
gcggaggagctggtggtaacgaagtc

SEQ ID NO: 9 - DNA, 26 bp, Artificial Sequence
  Primer for addition of  linker to GID1b cDNA
gcctccaccaggagtaagaagcacag

SEQ ID NO: 10 - DNA, 59 bp, Artificial Sequence
  Primer for Addition of linker to N-terminal domain of firefly luciferase
ctgtgcttcttactcctggtggaggcggaggcggaggcgaagacgccaaaaacataaag

SEQ ID NO: 11 - DNA, 19 bp, Artificial Sequence
  Primer for amplification of N-terminal domain of firefly luciferase
ttatccatccttgtcaatc

SEQ ID NO: 12 - DNA, 2778 bp, Artificial
  GID1C-sensor nucleotide sequence
atgtccggttatgtaaacaatccggaagcgaccaacgccttgattgacaaggatggatggctacattctggagacatagcttactgggacgaagacgaacacttcttcatcgttgaccgcctgaagtctctgattaagtacaaaggctatcaggtggctcccgctgaattggaatccatcttgctccaacaccccaacatcttcgacgcaggtgtcgcaggtcttcccgacgatgacgccggtgaacttcccgccgccgttgttgttttggagcacggaaagacgatgacggaaaaagagatcgtggattacgtcgccagtcaagtaacaaccgcgaaaaagttgcgcggaggagttgtgtttgtggacgaagtaccgaaaggtcttaccggaaaactcgacgcaagaaaaatcagagagatcctcataaaggccaagaagggcggaaagatcgccgtgggtggcgggggtggcggaggagctggaagtgaagaagttaatcttattgagagcaagacagtggttcctctcaatacatgggttctaatatccaactttaagctagcttacaatctcctgcgtcgccctgacggaacttttaaccgtcatctcgcagagtttctagaccggaaagtccctgcaaatgccaaccctgttaatggggtcttctcttttgatgtgatcatcgatcgccaaactaatttgcttagcagagtttacagaccagctgatgctggcacttcaccaagtattactgatctacagaatcctgttgatggtgaaatagtgcctgttattgtcttctttcatggtggaagctttgcacattcttctgcaaacagtgctatttatgatactctttgtcgtaggcttgttggtttgtgtggtgctgttgttgtctctgtgaattatcgtcgtgcaccagagaatcgatacccttgtgcttatgatgatggatgggctgttttgaaatgggtcaactcgagttcttggcttagaagcaagaaagactcaaaggttcgtattttcttggcgggtgatagctctgggggtaacattgtgcataatgtcgcggtaagagcggttgagtcaaggatcgatgttttggggaacattttgcttaaccctatgtttggagggaccgaaagaacggaatctgagaaacgtttggatgggaagtactttgttacggttagagaccgagattggtattggagagcgtttcttcctgagggtgaagacagagagcatccagcgtgtagcccgtttggcccgagaagcaagagtctagaagggttgagtttccccaagagtcttgtcgttgtagcgggtttagatttgattcaagattggcaattgaagtacgcggaagggctcaagaaagcgggtcaagaggtgaagcttctttacttggagcaagccactattggcttctacttattgcctaacaacaatcacttccataccgttatggatgagatagctgcatttgtaaacgcagaatgccaaggtggaggcggaggcggaggcgaagacgccaaaaacataaagaaaggcccggcgccattctatccgctggaagatggaaccgctggagagcaactgcataaggctatgaagagatacgccctggttcctggaacaattgcttttacagatgcacatatcgaggtggacatcacttacgctgagtacttcgaaatgtccgttcggttggcagaagctatgaaacgatatgggctgaatacaaatcacagaatcgtcgtatgcagtgaaaactctcttcaattctttatgccggtgttgggcgcgttatttatcggagttgcagttgcgcccgcgaacgacatttataatgaacgtgaattgctcaacagtatgggcatttcgcagcctaccgtggtgttcgtttccaaaaaggggttgcaaaaaattttgaacgtgcaaaaaaagctcccaatcatccaaaaaattattatcatggattctaaaacggattaccagggatttcagtcgatgtacacgttcgtcacatctcatctacctcccggttttaatgaatacgattttgtgccagagtccttcgatagggacaagacaattgcactgatcatgaactcctctggatctactggtctgcctaaaggtgtcgctctgcctcatagaactgcctgcgtgagattctcgcatgccagagatcctatttttggcaatcaaatcattccggatactgcgattttaagtgttgttccattccatcacggttttggaatgtttactacactcggatatttgatatgtggatttcgagtcgtcttaatgtatagatttgaagaagagctgtttctgaggagccttcaggattacaagattcaaagtgcgctgctggtgccaaccctattctccttcttcgccaaaagcactctgattgacaaatacgatttatctaatttacacgaaattgcttctggtggcgctcccctctctaaggaagtcggggaagcggttgccaagaggttccatctgccaggtatcaggcaaggatatgggctcactgagactacatcagctattctgattacacccgagggggatgataaaccgggcgcggtcggtaaagttgttccattttttgaagcgaaggttgtggatctggataccgggaaaacgctgggcgttaatcaaagaggcgaactgtgtgtgagaggtcctatgattatgtccggttatgtaaacaatccggaagcgaccaacgccttgattgacaaggatggataa

SEQ ID NO: 13 - protein, 925 aa, Artificial
  GID1C sensor peptide
MSGYVNNPEATNALIDKDGWLHSGDIAYWDEDEHFFIVDRLKSLIKYKGYQVAPAELESILLQHPNIFDAGVAGLPDDDAGELPAAVVVLEHGKTMTEKEIVDYVASQVTTAKKLRGGVVFVDEVPKGLTGKLDARKIREILIKAKKGGKIAVGGGGGGGAGSEEVNLIESKTVVPLNTWVLISNFKLAYNLLRRPDGTFNRHLAEFLDRKVPANANPVNGVFSFDVIIDRQTNLLSRVYRPADAGTSPSITDLQNPVDGEIVPVIVFFHGGSFAHSSANSAIYDTLCRRLVGLCGAVVVSVNYRRAPENRYPCAYDDGWAVLKWVNSSSWLRSKKDSKVRIFLAGDSSGGNIVHNVAVRAVESRIDVLGNILLNPMFGGTERTESEKRLDGKYFVTVRDRDWYWRAFLPEGEDREHPACSPFGPRSKSLEGLSFPKSLVVVAGLDLIQDWQLKYAEGLKKAGQEVKLLYLEQATIGFYLLPNNNHFHTVMDEIAAFVNAECQGGGGGGGEDAKNIKKGPAPFYPLEDGTAGEQLHKAMKRYALVPGTIAFTDAHIEVDITYAEYFEMSVRLAEAMKRYGLNTNHRIVVCSENSLQFFMPVLGALFIGVAVAPANDIYNERELLNSMGISQPTVVFVSKKGLQKILNVQKKLPIIQKIIIMDSKTDYQGFQSMYTFVTSHLPPGFNEYDFVPESFDRDKTIALIMNSSGSTGLPKGVALPHRTACVRFSHARDPIFGNQIIPDTAILSVVPFHHGFGMFTTLGYLICGFRVVLMYRFEEELFLRSLQDYKIQSALLVPTLFSFFAKSTLIDKYDLSNLHEIASGGAPLSKEVGEAVAKRFHLPGIRQGYGLTETTSAILITPEGDDKPGAVGKVVPFFEAKVVDLDTGKTLGVNQRGELCVRGPMIMSGYVNNPEATNALIDKDG

SEQ ID NO: 14 - DNA, 26 bp, Artificial Sequence
  Primer for amplification of GID1c cDNA
atggctggaagtgaagaagttaatct

SEQ ID NO: 15 - DNA, 21 bp, Artificial Sequence
  Primer for amplification of GID1c cDNA
tcattggcattctgcgtttac

SEQ ID NO: 16 - DNA, 57 bp, Artificial Sequence
  Primer for Addition of linker to C-terminal domain of firefly luciferase
gattaacttcttcacttccagctcctccgccacccccgccacccacggcgatctttc

SEQ ID NO: 17 - DNA, 31 bp, Artificial Sequence
  Primer for Addition of linker to GID1c cDNA
ggcggaggagctggaagtgaagaagttaatc

SEQ ID NO: 18 - DNA, 27 bp, Artificial Sequence
  Primer for Addition of linker to GID1c cDNA
gcctccaccttggcattctgcgtttac

SEQ ID NO: 19 - DNA, 54 bp, Artificial Sequence
  Primer for Addition of linker to N-terminal domain firefly luciferase
gtaaacgcagaatgccaaggtggaggcggaggcggaggcgaagacgccaaaaac

SEQ ID NO: 20 - DNA, 21 bp, Artificial Sequence
  Primer for amplification of N-terminal domain of firefly luciferase being non-overlapping
ttaaatcataggacctctcac

SEQ ID NO: 21 - DNA, 21 bp, Artificial Sequence
  Primer for introduction of V53A mutation into GID1b by PCR amplification
ccgtaaagcccccgccaactc

SEQ ID NO: 22 - DNA, 25 bp, Artificial Sequence
  Primer for Introduction of V53A mutation into GID1b by PCR amplification
ggcgggggctttacggtcaaggaac

SEQ ID NO: 23 - DNA, 19 bp, Artificial Sequence
  Primer for DELLA protein GAI gene PCR amplification, without ATG
aagagagatcatcatcatc

SEQ ID NO: 24 - DNA, 23 bp, Artificial Sequence
  Primer for DELLA protein GAI gene PCR amplification
ctaattggtggagagtttccaag

SEQ ID NO: 25 - DNA, 2820 bp, Artificial Sequence
  GID1B.5 sensor nucleotide sequence
atgtccggttatgtaaacaatccggaagcgaccaacgccttgattgacaaggatggatggctacattctggagacatagcttactgggacgaagacgaacacttcttcatcgttgaccgcctgaagtctctgattaagtacaaaggctatcaggtggctcccgctgaattggaatccatcttgctccaacaccccaacatcttcgacgcaggtgtcgcaggtcttcccgacgatgacgccggtgaacttcccgccgccgttgttgttttggagcacggaaagacgatgacggaaaaagagatcgtggattacgtcgccagtcaagtaacaaccgcgaaaaagttgcgcggaggagttgtgtttgtggacgaagtaccgaaaggtcttaccggaaaactcgacgcaagaaaaatcagagagatcctcataaaggccaagaagggcggaaagatcgccgtgggtggcgggggtggcggaggagctggtggtaacgaagtcaaccttaacgaatgcaagagaattgtcccactcaacacatgggtcctcatttccaatttcaagcttgcttacaaagtcctccgtcgccctgacggttctttcaaccgcgacctcgccgagttccttgaccgtaaagcccccgccaactctttccccctcgacggcgttttctccttcgaccacgtcgactcaacaactaaccttctcaccagaatctaccaacctgcgtctctccttcatcagacccgtcacggaaccctcgagctaaccaaacctctcagtactacagagatcgtccctgttctcattttcttccatggaggcagcttcactcattcctccgccaatagtgctatctacgacactttctgccgacgccttgtcaccatttgcggtgttgttgttgtctctgttgattaccggagatcccctgagcatcgctacccttgtgcttacgacgatggatggaacgctctcaactgggtcaagtccagagtctggcttcagagtggtaaagactccaatgtttatgtttatttggctggagatagctctggaggcaacattgctcacaatgtcgctgtcagagctaccaatgaaggagtcaaagtgttggggaacattcttcttcatccaatgtttggtggacaggagaggactcagtctgagaagacccttgatggcaaatactttgtgactatacaagatcgagattggtattggagggcttatctaccggaaggtgaagatagagatcatccagcatgtaatccctttggcccgagaggtcaaagccttaaaggagtcaactttccaaagagtcttgttgttgtcgctggtttagatcttgttcaagattggcaattagcctatgtggatgggcttaagaagactggtcttgaagtcaatcttttgtatttgaaacaagctaccattggcttttacttcttgcctaacaatgatcactttcattgtcttatggaagagttgaataagtttgtgcactccatagaggattctcaaagcaagtcaagtcctgtgcttcttactcctggtggaggcggaggcggaggcgaagacgccaaaaacataaagaaaggcccggcgccattctatccgctggaagatggaaccgctggagagcaactgcataaggctatgaagagatacgccctggttcctggaacaattgcttttacagatgcacatatcgaggtggacatcacttacgctgagtacttcgaaatgtccgttcggttggcagaagctatgaaacgatatgggctgaatacaaatcacagaatcgtcgtatgcagtgaaaactctcttcaattctttatgccggtgttgggcgcgttatttatcggagttgcagttgcgcccgcgaacgacatttataatgaacgtgaattgctcaacagtatgggcatttcgcagcctaccgtggtgttcgtttccaaaaaggggttgcaaaaaattttgaacgtgcaaaaaaagctcccaatcatccaaaaaattattatcatggattctaaaacggattaccagggatttcagtcgatgtacacgttcgtcacatctcatctacctcccggttttaatgaatacgattttgtgccagagtccttcgatagggacaagacaattgcactgatcatgaactcctctggatctactggtctgcctaaaggtgtcgctctgcctcatagaactgcctgcgtgagattctcgcatgccagagatcctatttttggcaatcaaatcattccggatactgcgattttaagtgttgttccattccatcacggttttggaatgtttactacactcggatatttgatatgtggatttcgagtcgtcttaatgtatagatttgaagaagagctgtttctgaggagccttcaggattacaagattcaaagtgcgctgctggtgccaaccctattctccttcttcgccaaaagcactctgattgacaaatacgatttatctaatttacacgaaattgcttctggtggcgctcccctctctaaggaagtcggggaagcggttgccaagaggttccatctgccaggtatcaggcaaggatatgggctcactgagactacatcagctattctgattacacccgagggggatgataaaccgggcgcggtcggtaaagttgttccattttttgaagcgaaggttgtggatctggataccgggaaaacgctgggcgttaatcaaagaggcgaactgtgtgtgagaggtcctatgattatgtccggttatgtaaacaatccggaagcgaccaacgccttgattgacaaggatggataa

SEQ ID NO: 26 - protein, 939 aa, Artificial Sequence
  GID1B.5 sensor protein sequence
MSGYVNNPEATNALIDKDGWLHSGDIAYWDEDEHFFIVDRLKSLIKYKGYQVAPAELESILLQHPNIFDAGVAGLPDDDAGELPAAVVVLEHGKTMTEKEIVDYVASQVTTAKKLRGGVVFVDEVPKGLTGKLDARKIREILIKAKKGGKIAVGGGGGGGAGGNEVNLNECKRIVPLNTWVLISNFKLAYKVLRRPDGSFNRDLAEFLDRKAPANSFPLDGVFSFDHVDSTTNLLTRIYQPASLLHQTRHGTLELTKPLSTTEIVPVLIFFHGGSFTHSSANSAIYDTFCRRLVTICGVVVVSVDYRRSPEHRYPCAYDDGWNALNWVKSRVWLQSGKDSNVYVYLAGDSSGGNIAHNVAVRATNEGVKVLGNILLHPMFGGQERTQSEKTLDGKYFVTIQDRDWYWRAYLPEGEDRDHPACNPFGPRGQSLKGVNFPKSLVVVAGLDLVQDWQLAYVDGLKKTGLEVNLLYLKQATIGFYFLPNNDHFHCLMEELNKFVHSIEDSQSKSSPVLLTPGGGGGGGEDAKNIKKGPAPFYPLEDGTAGEQLHKAMKRYALVPGTIAFTDAHIEVDITYAEYFEMSVRLAEAMKRYGLNTNHRIVVCSENSLQFFMPVLGALFIGVAVAPANDIYNERELLNSMGISQPTVVFVSKKGLQKILNVQKKLPIIQKIIIMDSKTDYQGFQSMYTFVTSHLPPGFNEYDFVPESFDRDKTIALIMNSSGSTGLPKGVALPHRTACVRFSHARDPIFGNQIIPDTAILSVVPFHHGFGMFTTLGYLICGFRVVLMYRFEEELFLRSLQDYKIQSALLVPTLFSFFAKSTLIDKYDLSNLHEIASGGAPLSKEVGEAVAKRFHLPGIRQGYGLTETTSAILITPEGDDKPGAVGKVVPFFEAKVVDLDTGKTLGVNQRGELCVRGPMIMSGYVNNPEATNALIDKDG